European Patent Application EP 4 779 003 A1, published July 22, 2026. Title: WATER-SOLUBLE AUTOMATIC DISHWASHING DETERGENT POUCH. Applicant: The Procter & Gamble Company. The sequence listing filed with the application follows.

SEQUENCE LISTING (3 sequences)

SEQ ID NO: 1 - protein, 269 aa, Bacillus gibsonii
QQTVPWGITRVQAPAVHNRGITGSGVRVAILDSGISAHSDLNIRGGASFVPGEPTTADLNGHGTHVAGTVAALNNSIGVIGVAPNAELYAVKVLGANGSGSVSGIAQGLEWAATNNMHIANMSLGSDFPSSTLERAVNYATSRDVLVIAATGNNGSGSVGYPARYANAMAVGATDQNNRRANFSQYGTGIDIVAPGVNVQSTYPGNRYVSMNGTSMATPHVAGAAALVKQRYPSWNATQIRNHLKNTATNLGNSSQFGSGLVNAEAATR

SEQ ID NO: 2 - protein, 269 aa, Bacillus gibsonii [sequence omitted]

SEQ ID NO: 3 - protein, 484 aa, synthetic construct
  REGION 1..484: note = Synthetic construct
HHNGTNGTMMQYFEWHLPNDGQHWNRLRNDAANLKNLGINAVWIPPAWKGTSQNDVGYGAYDLYDLGEFNQKGTIRTKYGTRSQLQSAIARLQNNGIQVFGDVVMNHKGGADGTERVQAVEVNPSNRNQEVTGEYTIEAWTKFDFPGRGNTHSSFKWRWYHFDGTDWDQSRNLNNRIYKFTGKAWDWEVDTENGNYDYLMYADVDMDHPEVINELRRWGVWYTNTLNLDGFRIDAVKHIKYQFTRDWLNHVRSTTGKNNMFAVAEFWKNDLGAIENYLSKTNWNHSVFDVPLHYNLYNASKSGGNYDMRQILNGTVVSKHPIHAVTFVDNHDSQPAEALESFVEAWFKPLAYALILTREQGYPSVFYGDYYGIPTHGVAAMKGKIDPILEARQKYAYGTQHDYLDHHNIIGWTREGNSAHPNSGLATIMSDGPGGSKWMYVGRHKAGQVWRDITGNRTGTVTINADGWGNFSVNGGSVSIWVNK